European Patent Application EP 4 349 992 A1, published April 10, 2024. Title: Cells sensitive to botulinum toxin via lentivirus-mediated genomic integration. Applicant: ATGC CO., LTD. The sequence listing filed with the application follows.

SEQUENCE LISTING (12 sequences)

SEQ ID NO: 1 - DNA, 17 bp, Artificial Sequence
  SEPTIN2 V2
agagctcgtttagtgaa

SEQ ID NO: 2 - DNA, 20 bp, Artificial Sequence
  SEPTIN2-600F
ggatgaaattgaagaacata

SEQ ID NO: 3 - DNA, 17 bp, Artificial Sequence
  TXN V2
agagctcgtttagtgaa

SEQ ID NO: 4 - DNA, 18 bp, Artificial Sequence
  TXN forward
cttttcaggaagccttgg

SEQ ID NO: 5 - DNA, 18 bp, Artificial Sequence
  SEPTIN2 forward
gtctaagcaacagccaac

SEQ ID NO: 6 - DNA, 19 bp, Artificial Sequence
  DDK reverse
cttatcgtcgtcatccttg

SEQ ID NO: 7 - DNA, 20 bp, Artificial Sequence
  GH20
gaagagccaaggacaggtac

SEQ ID NO: 8 - DNA, 21 bp, Artificial Sequence
  GH21
ggaaaatagaccaataggcag

SEQ ID NO: 9 - protein, 361 aa, Homo sapiens
MSKQQPTQFINPETPGYVGFANLPNQVHRKSVKKGFEFTLMVVGESGLGKSTLINSLFLTDLYPERVIPGAAEKIERTVQIEASTVEIEERGVKLRLTVVDTPGYGDAINCRDCFKTIISYIDEQFERYLHDESGLNRRHIIDNRVHCCFYFISPFGHGLKPLDVAFMKAIHNKVNIVPVIAKADTLTLKERERLKKRILDEIEEHNIKIYHLPDAESDEDEDFKEQTRLLKASIPFSVVGSNQLIEAKGKKVRGRLYPWGVVEVENPEHNDFLKLRTMLITHMQDLQEVTQDLHYENFRSERLKRGGRKVENEDMNKDQILLEKEAELRRMQEMIARMQAQMQMQMQGGDGDGGALGHHV

SEQ ID NO: 10 - DNA, 8138 bp, Artificial Sequence
  SEPTIN2 expression construct sequence
gtcgacggatcgggagatctcccgatcccctatggtgcactctcagtacaatctgctctgatgccgcatagttaagccagtatctgctccctgcttgtgtgttggaggtcgctgagtagtgcgcgagcaaaatttaagctacaacaaggcaaggcttgaccgacaattgcatgaagaatctgcttagggttaggcgttttgcgctgcttcgcgatgtacgggccagatatcgcgttgacattgattattgactagttattaatagtaatcaattacggggtcattagttcatagcccatatatggagttccgcgttacataacttacggtaaatggcccgcctggctgaccgcccaacgacccccgcccattgacgtcaataatgacgtatgttcccatagtaacgccaatagggactttccattgacgtcaatgggtggagtatttacggtaaactgcccacttggcagtacatcaagtgtatcatatgccaagtacgccccctattgacgtcaatgacggtaaatggcccgcctggcattatgcccagtacatgaccttatgggactttcctacttggcagtacatctacgtattagtcatcgctattaccatggtgatgcggttttggcagtacatcaatgggcgtggatagcggtttgactcacggggatttccaagtctccaccccattgacgtcaatgggagtttgttttggcaccaaaatcaacgggactttccaaaatgtcgtaacaactccgccccattgacgcaaatgggcggtaggcgtgtacggtgggaggtctatataagcagcgcgttttgcctgtactgggtctctctggttagaccagatctgagcctgggagctctctggctaactagggaacccactgcttaagcctcaataaagcttgccttgagtgcttcaagtagtgtgtgcccgtctgttgtgtgactctggtaactagagatccctcagacccttttagtcagtgtggaaaatctctagcagtggcgcccgaacagggacttgaaagcgaaagggaaaccagaggagctctctcgacgcaggactcggcttgctgaagcgcgcacggcaagaggcgaggggcggcgactggtgagtacgccaaaaattttgactagcggaggctagaaggagagagatgggtgcgagagcgtcagtattaagcgggggagaattagatcgcgatgggaaaaaattcggttaaggccagggggaaagaaaaaatataaattaaaacatatagtatgggcaagcagggagctagaacgattcgcagttaatcctggcctgttagaaacatcagaaggctgtagacaaatactgggacagctacaaccatcccttcagacaggatcagaagaacttagatcattatataatacagtagcaaccctctattgtgtgcatcaaaggatagagataaaagacaccaaggaagctttagacaagatagaggaagagcaaaacaaaagtaagaccaccgcacagcaagcggccggccgctgatcttcagacctggaggaggagatatgagggacaattggagaagtgaattatataaatataaagtagtaaaaattgaaccattaggagtagcacccaccaaggcaaagagaagagtggtgcagagagaaaaaagagcagtgggaataggagctttgttccttgggttcttgggagcagcaggaagcactatgggcgcagcgtcaatgacgctgacggtacaggccagacaattattgtctggtatagtgcagcagcagaacaatttgctgagggctattgaggcgcaacagcatctgttgcaactcacagtctggggcatcaagcagctccaggcaagaatcctggctgtggaaagatacctaaaggatcaacagctcctggggatttggggttgctctggaaaactcatttgcaccactgctgtgccttggaatgctagttggagtaataaatctctggaacagatttggaatcacacgacctggatggagtgggacagagaaattaacaattacacaagcttaatacactccttaattgaagaatcgcaaaaccagcaagaaaagaatgaacaagaattattggaattagataaatgggcaagtttgtggaattggtttaacataacaaattggctgtggtatataaaattattcataatgatagtaggaggcttggtaggtttaagaatagtttttgctgtactttctatagtgaatagagttaggcagggatattcaccattatcgtttcagacccacctcccaaccccgaggggacccgacaggcccgaaggaatagaagaagaaggtggagagagagacagagacagatccattcgattagtgaacggatcggcactgcgtgcgccaattctgcagacaaatggcagtattcatccacaattttaaaagaaaaggggggattggggggtacagtgcaggggaaagaatagtagacataatagcaacagacatacaaactaaagaattacaaaaacaaattacaaaaattcaaaattttcgggtttattacagggacagcagagatccagtttggttagtaccgggcccgctctagacatgtccaatatgaccgccatgttgacattgattattgactagttattaatagtaatcaattacggggtcattagttcatagcccatatatggagttccgcgttacataacttacggtaaatggcccgcctggctgaccgcccaacgacccccgcccattgacgtcaataatgacgtatgttcccatagtaacgccaatagggactttccattgacgtcaatgggtggagtatttacggtaaactgcccacttggcagtacatcaagtgtatcatatgccaagtccgccccctattgacgtcaatgacggtaaatggcccgcctggcattatgcccagtacatgaccttacgggactttcctacttggcagtacatctacgtattagtcatcgctattaccatggtgatgcggttttggcagtacaccaatgggcgtggatagcggtttgactcacggggatttccaagtctccaccccattgacgtcaatgggagtttgttttggcaccaaaatcaacgggactttccaaaatgtcgtaataaccccgccccgttgacgcaaatgggcggtaggcgtgtacggtgggaggtctatataagcagagctcgtttagtgaaccgtcagaattttgtaatacgactcactatagggcggccgggaattcgtcgactggatccggtaccgaggagatctgccgccgcgatcgccatgtctaagcaacagccaactcagtttataaatccagaaacacctggctatgttggatttgcaaacctccccaatcaagttcaccgaaaatcagtgaaaaaaggttttgagttcacactgatggtggtcggtgaatcaggtctaggaaaatcgactctcataaacagcctattcctaactgatctgtacccagaaagagtcatacctggagcagcagaaaaaattgaaagaactgtccagattgaggcttcaactgttgaaattgaagagcgaggggtcaagctacgcctgacagtggtagatacccctggctatggtgacgctatcaactgcagagattgttttaagacaattatctcctatattgatgagcaatttgagaggtacctgcatgacgagagcggcttgaacaggcggcacatcattgataatagggtgcattgttgcttttactttatttcaccttttggacatggacttaagcccttagatgtggcgtttatgaaggcaatacacaacaaggtgaatattgtgcctgtcattgcaaaagctgacactctcaccctgaaggaacgggagcggctgaagaaaaggattctggatgaaattgaagaacataacatcaaaatctatcacttacctgatgcagaatcagatgaagatgaagattttaaagagcagactagacttctcaaggctagcatcccattctctgtggttggatccaatcagttgattgaagccaaaggaaagaaggtcagaggccgcctctacccctggggtgttgtggaagtggagaacccagagcacaatgactttctgaagctgagaaccatgctcatcacccacatgcaggatctccaggaggtgacccaggaccttcattatgaaaacttccgttctgagagactcaagagaggcggcaggaaagtggagaatgaggacatgaataaagaccagatcttgctggaaaaagaagctgagctccgccgcatgcaagagatgattgcaaggatgcaggcgcagatgcagatgcagatgcagggcggggatggcgatggcggggctctcgggcaccacgtgacgcgtacgcggccgctcgagcagaaactcatctcagaagaggatctggcagcaaatgatatcctggattacaaggatgacgacgataaggtttgggtaggaagcggagctactaacttcagcctgctgaagcaggctggagacgtggaggagaaccctggacctatgaccgagtacaagcccacggtgcgcctcgccacccgcgacgacgtccccagggccgtacgcaccctcgccgccgcgttcgccgactaccccgccacgcgccacaccgtcgatccggatcgccacatcgagcgggtcaccgagctgcaagaactcttcctcacgcgcgtcgggctcgacatcggcaaggtgtgggtcgcggacgacggcgccgcggtggcggtctggaccacgccggagagcgtcgaagcgggggcggtgttcgccgagatcggcccgcgcatggccgagttgagcggttcccggctggccgcgcagcaacagatggaaggcctcctggcgccgcaccggcccaaggagcccgcgtggttcctggccaccgtcggcgtctcgcccgaccaccagggcaagggtctgggcagcgccgtcgtgctccccggagtggaggcggccgagcgcgccggggtgcccgccttcctggagacctccgcgccccgcaacctccccttctacgagcggctcggcttcaccgtcaccgccgacgtcgaggtgcccgaaggaccgcgcacctggtgcatgacccgcaagcccggtgcctgatgtacacccaaacggccggccgcggtctgtacaagtaggattcgtcgagggacctaataacttcgtatagcatacattatacgaagttatacatgtttaagggttccggttccactaggtacaattcgatatcaagcttatcgataatcaacctctggattacaaaatttgtgaaagattgactggtattcttaactatgttgctccttttacgctatgtggatacgctgctttaatgcctttgtatcatgctattgcttcccgtatggctttcattttctcctccttgtataaatcctggttgctgtctctttatgaggagttgtggcccgttgtcaggcaacgtggcgtggtgtgcactgtgtttgctgacgcaacccccactggttggggcattgccaccacctgtcagctcctttccgggactttcgctttccccctccctattgccacggcggaactcatcgccgcctgccttgcccgctgctggacaggggctcggctgttgggcactgacaattccgtggtgttgtcggggaaatcatcgtcctttccttggctgctcgcctgtgttgccacctggattctgcgcgggacgtccttctgctacgtcccttcggccctcaatccagcggaccttccttcccgcggcctgctgccggctctgcggcctcttccgcgtcttcgccttcgccctcagacgagtcggatctccctttgggccgcctccccgcatcgataccgtcgacctcgatcgagacctagaaaaacatggagcaatcacaagtagcaatacagcagctaccaatgctgattgtgcctggctagaagcacaagaggaggaggaggtgggttttccagtcacacctcaggtacctttaagaccaatgacttacaaggcagctgtagatcttagccactttttaaaagaaaaggggggactggaagggctaattcactcccaacgaagacaagatatccttgatctgtggatctaccacacacaaggctacttccctgattggcagaactacacaccagggccagggatcagatatccactgacctttggatggtgctacaagctagtaccagttgagcaagagaaggtagaagaagccaatgaaggagagaacacccgcttgttacaccctgtgagcctgcatgggatggatgacccggagagagaagtattagagtggaggtttgacagccgcctagcatttcatcacatggcccgagagctgcatccggactgtactgggtctctctggttagaccagatctgagcctgggagctctctggctaactagggaacccactgcttaagcctcaataaagcttgccttgagtgcttcaagtagtgtgtgcccgtctgttgtgtgactctggtaactagagatccctcagacccttttagtcagtgtggaaaatctctagcagcatgtgagcaaaaggccagcaaaaggccaggaaccgtaaaaaggccgcgttgctggcgtttttccataggctccgcccccctgacgagcatcacaaaaatcgacgctcaagtcagaggtggcgaaacccgacaggactataaagataccaggcgtttccccctggaagctccctcgtgcgctctcctgttccgaccctgccgcttaccggatacctgtccgcctttctcccttcgggaagcgtggcgctttctcatagctcacgctgtaggtatctcagttcggtgtaggtcgttcgctccaagctgggctgtgtgcacgaaccccccgttcagcccgaccgctgcgccttatccggtaactatcgtcttgagtccaacccggtaagacacgacttatcgccactggcagcagccactggtaacaggattagcagagcgaggtatgtaggcggtgctacagagttcttgaagtggtggcctaactacggctacactagaagaacagtatttggtatctgcgctctgctgaagccagttaccttcggaaaaagagttggtagctcttgatccggcaaacaaaccaccgctggtagcggtggtttttttgtttgcaagcagcagattacgcgcagaaaaaaaggatctcaagaagatcctttgatcttttctacggggtctgacgctcagtggaacgaaaactcacgttaagggattttggtcatgattacgccccgccctgccactcatcgcagtactgttgtaattcattaagcattctgccgacatggaagccatcacaaacggcatgatgaacctgaatcgccagcggcatcagcaccttgtcgccttgcgtataatatttgcccatggtgaaaacgggggcgaagaagttgtccatattggccacgtttaaatcaaaactggtgaaactcacccagggattggctgagacgaaaaacatattctcaataaaccctttagggaaataggccaggttttcaccgtaacacgccacatcttgcgaatatatgtgtagaaactgccggaaatcgtcgtggtattcactccagagcgatgaaaacgtttcagtttgctcatggaaaacggtgtaacaagggtgaacactatcccatatcaccagctcaccgtctttcattgccatacggaactccggatgagcattcatcaggcgggcaagaatgtgaataaaggccggataaaacttgtgcttatttttctttacggtctttaaaaaggccgtaatatccagctgaacggtctggttataggtacattgagcaactgactgaaatgcctcaaaatgttctttacgatgccattgggatatatcaacggtggtatatccagtgatttttttctccatactcttcctttttcaatattattgaagcatttatcagggttattgtctcatgagcggatacatatttgaatgtatttagaaaaataaacaaataggggttccgcgcacatttccccgaaaagtgccacctgac

SEQ ID NO: 11 - protein, 105 aa, Homo sapiens
MVKQIESKTAFQEALDAAGDKLVVVDFSATWCGPCKMIKPFFHSLSEKYSNVIFLEVDVDDCQDVASECEVKCMPTFQFFKKGQKVGEFSGANKEKLEATINELV

SEQ ID NO: 12 - DNA, 7370 bp, Artificial Sequence
  Thioredoxin expression construct sequence
gtcgacggatcgggagatctcccgatcccctatggtgcactctcagtacaatctgctctgatgccgcatagttaagccagtatctgctccctgcttgtgtgttggaggtcgctgagtagtgcgcgagcaaaatttaagctacaacaaggcaaggcttgaccgacaattgcatgaagaatctgcttagggttaggcgttttgcgctgcttcgcgatgtacgggccagatatcgcgttgacattgattattgactagttattaatagtaatcaattacggggtcattagttcatagcccatatatggagttccgcgttacataacttacggtaaatggcccgcctggctgaccgcccaacgacccccgcccattgacgtcaataatgacgtatgttcccatagtaacgccaatagggactttccattgacgtcaatgggtggagtatttacggtaaactgcccacttggcagtacatcaagtgtatcatatgccaagtacgccccctattgacgtcaatgacggtaaatggcccgcctggcattatgcccagtacatgaccttatgggactttcctacttggcagtacatctacgtattagtcatcgctattaccatggtgatgcggttttggcagtacatcaatgggcgtggatagcggtttgactcacggggatttccaagtctccaccccattgacgtcaatgggagtttgttttggcaccaaaatcaacgggactttccaaaatgtcgtaacaactccgccccattgacgcaaatgggcggtaggcgtgtacggtgggaggtctatataagcagcgcgttttgcctgtactgggtctctctggttagaccagatctgagcctgggagctctctggctaactagggaacccactgcttaagcctcaataaagcttgccttgagtgcttcaagtagtgtgtgcccgtctgttgtgtgactctggtaactagagatccctcagacccttttagtcagtgtggaaaatctctagcagtggcgcccgaacagggacttgaaagcgaaagggaaaccagaggagctctctcgacgcaggactcggcttgctgaagcgcgcacggcaagaggcgaggggcggcgactggtgagtacgccaaaaattttgactagcggaggctagaaggagagagatgggtgcgagagcgtcagtattaagcgggggagaattagatcgcgatgggaaaaaattcggttaaggccagggggaaagaaaaaatataaattaaaacatatagtatgggcaagcagggagctagaacgattcgcagttaatcctggcctgttagaaacatcagaaggctgtagacaaatactgggacagctacaaccatcccttcagacaggatcagaagaacttagatcattatataatacagtagcaaccctctattgtgtgcatcaaaggatagagataaaagacaccaaggaagctttagacaagatagaggaagagcaaaacaaaagtaagaccaccgcacagcaagcggccggccgctgatcttcagacctggaggaggagatatgagggacaattggagaagtgaattatataaatataaagtagtaaaaattgaaccattaggagtagcacccaccaaggcaaagagaagagtggtgcagagagaaaaaagagcagtgggaataggagctttgttccttgggttcttgggagcagcaggaagcactatgggcgcagcgtcaatgacgctgacggtacaggccagacaattattgtctggtatagtgcagcagcagaacaatttgctgagggctattgaggcgcaacagcatctgttgcaactcacagtctggggcatcaagcagctccaggcaagaatcctggctgtggaaagatacctaaaggatcaacagctcctggggatttggggttgctctggaaaactcatttgcaccactgctgtgccttggaatgctagttggagtaataaatctctggaacagatttggaatcacacgacctggatggagtgggacagagaaattaacaattacacaagcttaatacactccttaattgaagaatcgcaaaaccagcaagaaaagaatgaacaagaattattggaattagataaatgggcaagtttgtggaattggtttaacataacaaattggctgtggtatataaaattattcataatgatagtaggaggcttggtaggtttaagaatagtttttgctgtactttctatagtgaatagagttaggcagggatattcaccattatcgtttcagacccacctcccaaccccgaggggacccgacaggcccgaaggaatagaagaagaaggtggagagagagacagagacagatccattcgattagtgaacggatcggcactgcgtgcgccaattctgcagacaaatggcagtattcatccacaattttaaaagaaaaggggggattggggggtacagtgcaggggaaagaatagtagacataatagcaacagacatacaaactaaagaattacaaaaacaaattacaaaaattcaaaattttcgggtttattacagggacagcagagatccagtttggttagtaccgggcccgctctagacatgtccaatatgaccgccatgttgacattgattattgactagttattaatagtaatcaattacggggtcattagttcatagcccatatatggagttccgcgttacataacttacggtaaatggcccgcctggctgaccgcccaacgacccccgcccattgacgtcaataatgacgtatgttcccatagtaacgccaatagggactttccattgacgtcaatgggtggagtatttacggtaaactgcccacttggcagtacatcaagtgtatcatatgccaagtccgccccctattgacgtcaatgacggtaaatggcccgcctggcattatgcccagtacatgaccttacgggactttcctacttggcagtacatctacgtattagtcatcgctattaccatggtgatgcggttttggcagtacaccaatgggcgtggatagcggtttgactcacggggatttccaagtctccaccccattgacgtcaatgggagtttgttttggcaccaaaatcaacgggactttccaaaatgtcgtaataaccccgccccgttgacgcaaatgggcggtaggcgtgtacggtgggaggtctatataagcagagctcgtttagtgaaccgtcagaattttgtaatacgactcactatagggcggccgggaattcgtcgactggatccggtaccgaggagatctgccgccgcgatcgccatggtgaagcagatcgagagcaagactgcttttcaggaagccttggacgctgcaggtgataaacttgtagtagttgacttctcagccacgtggtgtgggccttgcaaaatgatcaagcctttctttcattccctctctgaaaagtattccaacgtgatattccttgaagtagatgtggatgactgtcaggatgttgcttcagagtgtgaagtcaaatgcatgccaacattccagttttttaagaagggacaaaaggtgggtgaattttctggagccaataaggaaaagcttgaagccaccattaatgaattagtcacgcgtacgcggccgctcgagcagaaactcatctcagaagaggatctggcagcaaatgatatcctggattacaaggatgacgacgataaggtttgggtaggaagcggagctactaacttcagcctgctgaagcaggctggagacgtggaggagaaccctggacctatgaccgagtacaagcccacggtgcgcctcgccacccgcgacgacgtccccagggccgtacgcaccctcgccgccgcgttcgccgactaccccgccacgcgccacaccgtcgatccggatcgccacatcgagcgggtcaccgagctgcaagaactcttcctcacgcgcgtcgggctcgacatcggcaaggtgtgggtcgcggacgacggcgccgcggtggcggtctggaccacgccggagagcgtcgaagcgggggcggtgttcgccgagatcggcccgcgcatggccgagttgagcggttcccggctggccgcgcagcaacagatggaaggcctcctggcgccgcaccggcccaaggagcccgcgtggttcctggccaccgtcggcgtctcgcccgaccaccagggcaagggtctgggcagcgccgtcgtgctccccggagtggaggcggccgagcgcgccggggtgcccgccttcctggagacctccgcgccccgcaacctccccttctacgagcggctcggcttcaccgtcaccgccgacgtcgaggtgcccgaaggaccgcgcacctggtgcatgacccgcaagcccggtgcctgatgtacacccaaacggccggccgcggtctgtacaagtaggattcgtcgagggacctaataacttcgtatagcatacattatacgaagttatacatgtttaagggttccggttccactaggtacaattcgatatcaagcttatcgataatcaacctctggattacaaaatttgtgaaagattgactggtattcttaactatgttgctccttttacgctatgtggatacgctgctttaatgcctttgtatcatgctattgcttcccgtatggctttcattttctcctccttgtataaatcctggttgctgtctctttatgaggagttgtggcccgttgtcaggcaacgtggcgtggtgtgcactgtgtttgctgacgcaacccccactggttggggcattgccaccacctgtcagctcctttccgggactttcgctttccccctccctattgccacggcggaactcatcgccgcctgccttgcccgctgctggacaggggctcggctgttgggcactgacaattccgtggtgttgtcggggaaatcatcgtcctttccttggctgctcgcctgtgttgccacctggattctgcgcgggacgtccttctgctacgtcccttcggccctcaatccagcggaccttccttcccgcggcctgctgccggctctgcggcctcttccgcgtcttcgccttcgccctcagacgagtcggatctccctttgggccgcctccccgcatcgataccgtcgacctcgatcgagacctagaaaaacatggagcaatcacaagtagcaatacagcagctaccaatgctgattgtgcctggctagaagcacaagaggaggaggaggtgggttttccagtcacacctcaggtacctttaagaccaatgacttacaaggcagctgtagatcttagccactttttaaaagaaaaggggggactggaagggctaattcactcccaacgaagacaagatatccttgatctgtggatctaccacacacaaggctacttccctgattggcagaactacacaccagggccagggatcagatatccactgacctttggatggtgctacaagctagtaccagttgagcaagagaaggtagaagaagccaatgaaggagagaacacccgcttgttacaccctgtgagcctgcatgggatggatgacccggagagagaagtattagagtggaggtttgacagccgcctagcatttcatcacatggcccgagagctgcatccggactgtactgggtctctctggttagaccagatctgagcctgggagctctctggctaactagggaacccactgcttaagcctcaataaagcttgccttgagtgcttcaagtagtgtgtgcccgtctgttgtgtgactctggtaactagagatccctcagacccttttagtcagtgtggaaaatctctagcagcatgtgagcaaaaggccagcaaaaggccaggaaccgtaaaaaggccgcgttgctggcgtttttccataggctccgcccccctgacgagcatcacaaaaatcgacgctcaagtcagaggtggcgaaacccgacaggactataaagataccaggcgtttccccctggaagctccctcgtgcgctctcctgttccgaccctgccgcttaccggatacctgtccgcctttctcccttcgggaagcgtggcgctttctcatagctcacgctgtaggtatctcagttcggtgtaggtcgttcgctccaagctgggctgtgtgcacgaaccccccgttcagcccgaccgctgcgccttatccggtaactatcgtcttgagtccaacccggtaagacacgacttatcgccactggcagcagccactggtaacaggattagcagagcgaggtatgtaggcggtgctacagagttcttgaagtggtggcctaactacggctacactagaagaacagtatttggtatctgcgctctgctgaagccagttaccttcggaaaaagagttggtagctcttgatccggcaaacaaaccaccgctggtagcggtggtttttttgtttgcaagcagcagattacgcgcagaaaaaaaggatctcaagaagatcctttgatcttttctacggggtctgacgctcagtggaacgaaaactcacgttaagggattttggtcatgattacgccccgccctgccactcatcgcagtactgttgtaattcattaagcattctgccgacatggaagccatcacaaacggcatgatgaacctgaatcgccagcggcatcagcaccttgtcgccttgcgtataatatttgcccatggtgaaaacgggggcgaagaagttgtccatattggccacgtttaaatcaaaactggtgaaactcacccagggattggctgagacgaaaaacatattctcaataaaccctttagggaaataggccaggttttcaccgtaacacgccacatcttgcgaatatatgtgtagaaactgccggaaatcgtcgtggtattcactccagagcgatgaaaacgtttcagtttgctcatggaaaacggtgtaacaagggtgaacactatcccatatcaccagctcaccgtctttcattgccatacggaactccggatgagcattcatcaggcgggcaagaatgtgaataaaggccggataaaacttgtgcttatttttctttacggtctttaaaaaggccgtaatatccagctgaacggtctggttataggtacattgagcaactgactgaaatgcctcaaaatgttctttacgatgccattgggatatatcaacggtggtatatccagtgatttttttctccatactcttcctttttcaatattattgaagcatttatcagggttattgtctcatgagcggatacatatttgaatgtatttagaaaaataaacaaataggggttccgcgcacatttccccgaaaagtgccacctgac